European Patent Application EP 4 241 848 A2, published September 13, 2023. Title: TGF-BETA RECEPTOR TYPE II FUSION PROTEINS AND USES THEREOF. Applicant: Acceleron Pharma Inc. The sequence listing filed with the application follows.

SEQUENCE LISTING (66 sequences)

SEQ ID NO: 1 - protein, 567 aa, Homo sapiens
MGRGLLRGLWPLHIVLWTRIASTIPPHVQKSVNNDMIVTDNNGAVKFPQLCKFCDVRFSTCDNQKSCMSNCSITSICEKPQEVCVAVWRKNDENITLETVCHDPKLPYHDFILEDAASPKCIMKEKKKPGETFFMCSCSSDECNDNIIFSEEYNTSNPDLLLVIFQVTGISLLPPLGVAISVIIIFYCYRVNRQQKLSSTWETGKTRKLMEFSEHCAIILEDDRSDISSTCANNINHNTELLPIELDTLVGKGRFAEVYKAKLKQNTSEQFETVAVKIFPYEEYASWKTEKDIFSDINLKHENILQFLTAEERKTELGKQYWLITAFHAKGNLQEYLTRHVISWEDLRKLGSSLARGIAHLHSDHTPCGRPKMPIVHRDLKSSNILVKNDLTCCLCDFGLSLRLDPTLSVDDLANSGQVGTARYMAPEVLESRMNLENVESFKQTDVYSMALVLWEMTSRCNAVGEVKDYEPPFGSKVREHPCVESMKDNVLRDRGRPEIPSFWLNHQGIQMVCETLTECWDHDPEARLTAQCVAERFSELEHLDRLSGRSCSEEKIPEDGSLNTTK

SEQ ID NO: 2 - protein, 592 aa, Homo sapiens
MGRGLLRGLWPLHIVLWTRIASTIPPHVQKSDVEMEAQKDEIICPSCNRTAHPLRHINNDMIVTDNNGAVKFPQLCKFCDVRFSTCDNQKSCMSNCSITSICEKPQEVCVAVWRKNDENITLETVCHDPKLPYHDFILEDAASPKCIMKEKKKPGETFFMCSCSSDECNDNIIFSEEYNTSNPDLLLVIFQVTGISLLPPLGVAISVIIIFYCYRVNRQQKLSSTWETGKTRKLMEFSEHCAIILEDDRSDISSTCANNINHNTELLPIELDTLVGKGRFAEVYKAKLKQNTSEQFETVAVKIFPYEEYASWKTEKDIFSDINLKHENILQFLTAEERKTELGKQYWLITAFHAKGNLQEYLTRHVISWEDLRKLGSSLARGIAHLHSDHTPCGRPKMPIVHRDLKSSNILVKNDLTCCLCDFGLSLRLDPTLSVDDLANSGQVGTARYMAPEVLESRMNLENVESFKQTDVYSMALVLWEMTSRCNAVGEVKDYEPPFGSKVREHPCVESMKDNVLRDRGRPEIPSFWLNHQGIQMVCETLTECWDHDPEARLTAQCVAERFSELEHLDRLSGRSCSEEKIPEDGSLNTTK

SEQ ID NO: 3 - protein, 4 aa, synthetic construct
  REGION 1..4: note = Description of Artificial Sequence: Synthetic peptide
TGGG

SEQ ID NO: 4 - protein, 11 aa, synthetic construct
  REGION 1..11: note = Description of Artificial Sequence: Synthetic peptide
TGGGGSGGGGS

SEQ ID NO: 5 - protein, 16 aa, synthetic construct
  REGION 1..16: note = Description of Artificial Sequence: Synthetic peptide
TGGGGSGGGGSGGGGS

SEQ ID NO: 6 - protein, 21 aa, synthetic construct
  REGION 1..21: note = Description of Artificial Sequence: Synthetic peptide
TGGGGSGGGGSGGGGSGGGGS

SEQ ID NO: 7 - protein, 10 aa, synthetic construct
  REGION 1..10: note = Description of Artificial Sequence: Synthetic peptide
TGGGPKSCDK

SEQ ID NO: 8 - DNA, 1248 bp, synthetic construct
  misc_feature 1..1248: note = Description of Artificial Sequence: Synthetic polynucleotide
  source 1..1248: mol_type = other DNA
atggatgcaatgaagagagggctctgctgtgtgctgctgctgtgtggagcagtcttcgtttcgcccggcgccacgatcccaccgcacgttcagaagtcggatgtggaaatggaggcccagaaagatgaaatcatctgccccagctgtaataggactgcccatccactgagacatattaataacgacatgatagtcactgacaacaacggtgcagtcaagtttccacaactgtgtaaattttgtgatgtgagattttccacctgtgacaaccagaaatcctgcatgagcaactgcagcatcacctccatctgtgagaagccacaggaagtctgtgtggctgtatggagaaagaatgacgagaacataacactagagacagtttgccatgaccccaagctcccctaccatgactttattctggaagatgctgcttctccaaagtgcattatgaaggaaaaaaaaaagcctggtgagactttcttcatgtgttcctgtagctctgatgagtgcaatgacaacatcatcttctcagaagaatataacaccagcaatcctgacaccggtggtggaactcacacatgcccaccgtgcccagcacctgaactcctggggggaccgtcagtcttcctcttccccccaaaacccaaggacaccctcatgatctcccggacccctgaggtcacatgcgtggtggtggacgtgagccacgaagaccctgaggtcaagttcaactggtacgtggacggcgtggaggtgcataatgccaagacaaagccgcgggaggagcagtacaacagcacgtaccgtgtggtcagcgtcctcaccgtcctgcaccaggactggctgaatggcaaggagtacaagtgcaaggtctccaacaaagccctcccagcccccatcgagaaaaccatctccaaagccaaagggcagccccgagaaccacaggtgtacaccctgcccccatcccgggaggagatgaccaagaaccaggtcagcctgacctgcctggtcaaaggcttctatcccagcgacatcgccgtggagtgggagagcaatgggcagccggagaacaactacaagaccacgcctcccgtgctggactccgacggctccttcttcctctatagcaagctcaccgtggacaagagcaggtggcagcaggggaacgtcttctcatgctccgtgatgcatgaggctctgcacaaccactacacgcagaagagcctctccctgtctccgggtaaatga

SEQ ID NO: 9 - protein, 415 aa, synthetic construct
  REGION 1..415: note = Description of Artificial Sequence: Synthetic polypeptide
MDAMKRGLCCVLLLCGAVFVSPGATIPPHVQKSDVEMEAQKDEIICPSCNRTAHPLRHINNDMIVTDNNGAVKFPQLCKFCDVRFSTCDNQKSCMSNCSITSICEKPQEVCVAVWRKNDENITLETVCHDPKLPYHDFILEDAASPKCIMKEKKKPGETFFMCSCSSDECNDNIIFSEEYNTSNPDTGGGTHTCPPCPAPELLGGPSVFLFPPKPKDTLMISRTPEVTCVVVDVSHEDPEVKFNWYVDGVEVHNAKTKPREEQYNSTYRVVSVLTVLHQDWLNGKEYKCKVSNKALPAPIEKTISKAKGQPREPQVYTLPPSREEMTKNQVSLTCLVKGFYPSDIAVEWESNGQPENNYKTTPPVLDSDGSFFLYSKLTVDKSRWQQGNVFSCSVMHEALHNHYTQKSLSLSPGK

SEQ ID NO: 10 - DNA, 1284 bp, synthetic construct
  misc_feature 1..1284: note = Description of Artificial Sequence: Synthetic polynucleotide
  source 1..1284: mol_type = other DNA
atggatgcaatgaagagagggctctgctgtgtgctgctgctgtgtggagcagtcttcgtttcgcccggcgccacgatcccaccgcacgttcagaagtcggatgtggaaatggaggcccagaaagatgaaatcatctgccccagctgtaataggactgcccatccactgagacatattaataacgacatgatagtcactgacaacaacggtgcagtcaagtttccacaactgtgtaaattttgtgatgtgagattttccacctgtgacaaccagaaatcctgcatgagcaactgcagcatcacctccatctgtgagaagccacaggaagtctgtgtggctgtatggagaaagaatgacgagaacataacactagagacagtttgccatgaccccaagctcccctaccatgactttattctggaagatgctgcttctccaaagtgcattatgaaggaaaaaaaaaagcctggtgagactttcttcatgtgttcctgtagctctgatgagtgcaatgacaacatcatcttctcagaagaatataacaccagcaatcctgacaccggtggtggaggaagtggtggaggtggttctggaggtggtggaagtactcacacatgcccaccgtgcccagcacctgaactcctggggggaccgtcagtcttcctcttccccccaaaacccaaggacaccctcatgatctcccggacccctgaggtcacatgcgtggtggtggacgtgagccacgaagaccctgaggtcaagttcaactggtacgtggacggcgtggaggtgcataatgccaagacaaagccgcgggaggagcagtacaacagcacgtaccgtgtggtcagcgtcctcaccgtcctgcaccaggactggctgaatggcaaggagtacaagtgcaaggtctccaacaaagccctcccagcccccatcgagaaaaccatctccaaagccaaagggcagccccgagaaccacaggtgtacaccctgcccccatcccgggaggagatgaccaagaaccaggtcagcctgacctgcctggtcaaaggcttctatcccagcgacatcgccgtggagtgggagagcaatgggcagccggagaacaactacaagaccacgcctcccgtgctggactccgacggctccttcttcctctatagcaagctcaccgtggacaagagcaggtggcagcaggggaacgtcttctcatgctccgtgatgcatgaggctctgcacaaccactacacgcagaagagcctctccctgtctccgggtaaatga

SEQ ID NO: 11 - protein, 427 aa, synthetic construct
  REGION 1..427: note = Description of Artificial Sequence: Synthetic polypeptide
MDAMKRGLCCVLLLCGAVFVSPGATIPPHVQKSDVEMEAQKDEIICPSCNRTAHPLRHINNDMIVTDNNGAVKFPQLCKFCDVRFSTCDNQKSCMSNCSITSICEKPQEVCVAVWRKNDENITLETVCHDPKLPYHDFILEDAASPKCIMKEKKKPGETFFMCSCSSDECNDNIIFSEEYNTSNPDTGGGGSGGGGSGGGGSTHTCPPCPAPELLGGPSVFLFPPKPKDTLMISRTPEVTCVVVDVSHEDPEVKFNWYVDGVEVHNAKTKPREEQYNSTYRVVSVLTVLHQDWLNGKEYKCKVSNKALPAPIEKTISKAKGQPREPQVYTLPPSREEMTKNQVSLTCLVKGFYPSDIAVEWESNGQPENNYKTTPPVLDSDGSFFLYSKLTVDKSRWQQGNVFSCSVMHEALHNHYTQKSLSLSPGK

SEQ ID NO: 12 - DNA, 1299 bp, synthetic construct
  misc_feature 1..1299: note = Description of Artificial Sequence: Synthetic polynucleotide
  source 1..1299: mol_type = other DNA
atggatgcaatgaagagagggctctgctgtgtgctgctgctgtgtggagcagtcttcgtttcgcccggcgccacgatcccaccgcacgttcagaagtcggatgtggaaatggaggcccagaaagatgaaatcatctgccccagctgtaataggactgcccatccactgagacatattaataacgacatgatagtcactgacaacaacggtgcagtcaagtttccacaactgtgtaaattttgtgatgtgagattttccacctgtgacaaccagaaatcctgcatgagcaactgcagcatcacctccatctgtgagaagccacaggaagtctgtgtggctgtatggagaaagaatgacgagaacataacactagagacagtttgccatgaccccaagctcccctaccatgactttattctggaagatgctgcttctccaaagtgcattatgaaggaaaaaaaaaagcctggtgagactttcttcatgtgttcctgtagctctgatgagtgcaatgacaacatcatcttctcagaagaatataacaccagcaatcctgacaccggtggtggaggttctggaggtggaggaagtggtggaggtggttctggaggtggtggaagtactcacacatgcccaccgtgcccagcacctgaactcctggggggaccgtcagtcttcctcttccccccaaaacccaaggacaccctcatgatctcccggacccctgaggtcacatgcgtggtggtggacgtgagccacgaagaccctgaggtcaagttcaactggtacgtggacggcgtggaggtgcataatgccaagacaaagccgcgggaggagcagtacaacagcacgtaccgtgtggtcagcgtcctcaccgtcctgcaccaggactggctgaatggcaaggagtacaagtgcaaggtctccaacaaagccctcccagcccccatcgagaaaaccatctccaaagccaaagggcagccccgagaaccacaggtgtacaccctgcccccatcccgggaggagatgaccaagaaccaggtcagcctgacctgcctggtcaaaggcttctatcccagcgacatcgccgtggagtgggagagcaatgggcagccggagaacaactacaagaccacgcctcccgtgctggactccgacggctccttcttcctctatagcaagctcaccgtggacaagagcaggtggcagcaggggaacgtcttctcatgctccgtgatgcatgaggctctgcacaaccactacacgcagaagagcctctccctgtctccgggtaaatga

SEQ ID NO: 13 - protein, 432 aa, synthetic construct
  REGION 1..432: note = Description of Artificial Sequence: Synthetic polypeptide
MDAMKRGLCCVLLLCGAVFVSPGATIPPHVQKSDVEMEAQKDEIICPSCNRTAHPLRHINNDMIVTDNNGAVKFPQLCKFCDVRFSTCDNQKSCMSNCSITSICEKPQEVCVAVWRKNDENITLETVCHDPKLPYHDFILEDAASPKCIMKEKKKPGETFFMCSCSSDECNDNIIFSEEYNTSNPDTGGGGSGGGGSGGGGSGGGGSTHTCPPCPAPELLGGPSVFLFPPKPKDTLMISRTPEVTCVVVDVSHEDPEVKFNWYVDGVEVHNAKTKPREEQYNSTYRVVSVLTVLHQDWLNGKEYKCKVSNKALPAPIEKTISKAKGQPREPQVYTLPPSREEMTKNQVSLTCLVKGFYPSDIAVEWESNGQPENNYKTTPPVLDSDGSFFLYSKLTVDKSRWQQGNVFSCSVMHEALHNHYTQKSLSLSPGK

SEQ ID NO: 14 - DNA, 1269 bp, synthetic construct
  misc_feature 1..1269: note = Description of Artificial Sequence: Synthetic polynucleotide
  source 1..1269: mol_type = other DNA
atggatgcaatgaagagagggctctgctgtgtgctgctgctgtgtggagcagtcttcgtttcgcccggcgccacgatcccaccgcacgttcagaagtcggatgtggaaatggaggcccagaaagatgaaatcatctgccccagctgtaataggactgcccatccactgagacatattaataacgacatgatagtcactgacaacaacggtgcagtcaagtttccacaactgtgtaaattttgtgatgtgagattttccacctgtgacaaccagaaatcctgcatgagcaactgcagcatcacctccatctgtgagaagccacaggaagtctgtgtggctgtatggagaaagaatgacgagaacataacactagagacagtttgccatgaccccaagctcccctaccatgactttattctggaagatgctgcttctccaaagtgcattatgaaggaaaaaaaaaagcctggtgagactttcttcatgtgttcctgtagctctgatgagtgcaatgacaacatcatcttctcagaagaatataacaccagcaatcctgacaccggtggaggtggttctggaggtggtggaagtactcacacatgcccaccgtgcccagcacctgaactcctggggggaccgtcagtcttcctcttccccccaaaacccaaggacaccctcatgatctcccggacccctgaggtcacatgcgtggtggtggacgtgagccacgaagaccctgaggtcaagttcaactggtacgtggacggcgtggaggtgcataatgccaagacaaagccgcgggaggagcagtacaacagcacgtaccgtgtggtcagcgtcctcaccgtcctgcaccaggactggctgaatggcaaggagtacaagtgcaaggtctccaacaaagccctcccagcccccatcgagaaaaccatctccaaagccaaagggcagccccgagaaccacaggtgtacaccctgcccccatcccgggaggagatgaccaagaaccaggtcagcctgacctgcctggtcaaaggcttctatcccagcgacatcgccgtggagtgggagagcaatgggcagccggagaacaactacaagaccacgcctcccgtgctggactccgacggctccttcttcctctatagcaagctcaccgtggacaagagcaggtggcagcaggggaacgtcttctcatgctccgtgatgcatgaggctctgcacaaccactacacgcagaagagcctctccctgtctccgggtaaatga

SEQ ID NO: 15 - protein, 422 aa, synthetic construct
  REGION 1..422: note = Description of Artificial Sequence: Synthetic polypeptide
MDAMKRGLCCVLLLCGAVFVSPGATIPPHVQKSDVEMEAQKDEIICPSCNRTAHPLRHINNDMIVTDNNGAVKFPQLCKFCDVRFSTCDNQKSCMSNCSITSICEKPQEVCVAVWRKNDENITLETVCHDPKLPYHDFILEDAASPKCIMKEKKKPGETFFMCSCSSDECNDNIIFSEEYNTSNPDTGGGGSGGGGSTHTCPPCPAPELLGGPSVFLFPPKPKDTLMISRTPEVTCVVVDVSHEDPEVKFNWYVDGVEVHNAKTKPREEQYNSTYRVVSVLTVLHQDWLNGKEYKCKVSNKALPAPIEKTISKAKGQPREPQVYTLPPSREEMTKNQVSLTCLVKGFYPSDIAVEWESNGQPENNYKTTPPVLDSDGSFFLYSKLTVDKSRWQQGNVFSCSVMHEALHNHYTQKSLSLSPGK

SEQ ID NO: 16 - DNA, 1266 bp, synthetic construct
  misc_feature 1..1266: note = Description of Artificial Sequence: Synthetic polynucleotide
  source 1..1266: mol_type = other DNA
atggatgcaatgaagagagggctctgctgtgtgctgctgctgtgtggagcagtcttcgtttcgcccggcgccacgatcccaccgcacgttcagaagtcggatgtggaaatggaggcccagaaagatgaaatcatctgccccagctgtaataggactgcccatccactgagacatattaataacgacatgatagtcactgacaacaacggtgcagtcaagtttccacaactgtgtaaattttgtgatgtgagattttccacctgtgacaaccagaaatcctgcatgagcaactgcagcatcacctccatctgtgagaagccacaggaagtctgtgtggctgtatggagaaagaatgacgagaacataacactagagacagtttgccatgaccccaagctcccctaccatgactttattctggaagatgctgcttctccaaagtgcattatgaaggaaaaaaaaaagcctggtgagactttcttcatgtgttcctgtagctctgatgagtgcaatgacaacatcatcttctcagaagaatataacaccagcaatcctgacaccggtggtggacccaaatcttgtgacaaaactcacacatgcccaccgtgcccagcacctgaactcctggggggaccgtcagtcttcctcttccccccaaaacccaaggacaccctcatgatctcccggacccctgaggtcacatgcgtggtggtggacgtgagccacgaagaccctgaggtcaagttcaactggtacgtggacggcgtggaggtgcataatgccaagacaaagccgcgggaggagcagtacaacagcacgtaccgtgtggtcagcgtcctcaccgtcctgcaccaggactggctgaatggcaaggagtacaagtgcaaggtctccaacaaagccctcccagcccccatcgagaaaaccatctccaaagccaaagggcagccccgagaaccacaggtgtacaccctgcccccatcccgggaggagatgaccaagaaccaggtcagcctgacctgcctggtcaaaggcttctatcccagcgacatcgccgtggagtgggagagcaatgggcagccggagaacaactacaagaccacgcctcccgtgctggactccgacggctccttcttcctctatagcaagctcaccgtggacaagagcaggtggcagcaggggaacgtcttctcatgctccgtgatgcatgaggctctgcacaaccactacacgcagaagagcctctccctgtccccgggtaaatga

SEQ ID NO: 17 - protein, 421 aa, synthetic construct
  REGION 1..421: note = Description of Artificial Sequence: Synthetic polypeptide
MDAMKRGLCCVLLLCGAVFVSPGATIPPHVQKSDVEMEAQKDEIICPSCNRTAHPLRHINNDMIVTDNNGAVKFPQLCKFCDVRFSTCDNQKSCMSNCSITSICEKPQEVCVAVWRKNDENITLETVCHDPKLPYHDFILEDAASPKCIMKEKKKPGETFFMCSCSSDECNDNIIFSEEYNTSNPDTGGGPKSCDKTHTCPPCPAPELLGGPSVFLFPPKPKDTLMISRTPEVTCVVVDVSHEDPEVKFNWYVDGVEVHNAKTKPREEQYNSTYRVVSVLTVLHQDWLNGKEYKCKVSNKALPAPIEKTISKAKGQPREPQVYTLPPSREEMTKNQVSLTCLVKGFYPSDIAVEWESNGQPENNYKTTPPVLDSDGSFFLYSKLTVDKSRWQQGNVFSCSVMHEALHNHYTQKSLSLSPGK

SEQ ID NO: 18 - protein, 162 aa, synthetic construct
  REGION 1..162: note = Description of Artificial Sequence: Synthetic polypeptide
TIPPHVQKSDVEMEAQKDEIICPSCNRTAHPLRHINNDMIVTDNNGAVKFPQLCKFCDVRFSTCDNQKSCMSNCSITSICEKPQEVCVAVWRKNDENITLETVCHDPKLPYHDFILEDAASPKCIMKEKKKPGETFFMCSCSSDECNDNIIFSEEYNTSNPD

SEQ ID NO: 19 - protein, 5 aa, synthetic construct
  REGION 1..5: note = Description of Artificial Sequence: Synthetic peptide
GGGGS

SEQ ID NO: 20 - protein, 225 aa, synthetic construct
  REGION 1..225: note = Description of Artificial Sequence: Synthetic polypeptide
THTCPPCPAPELLGGPSVFLFPPKPKDTLMISRTPEVTCVVVDVSHEDPEVKFNWYVDGVEVHNAKTKPREEQYNSTYRVVSVLTVLHQDWLNGKEYKCKVSNKALPAPIEKTISKAKGQPREPQVYTLPPSREEMTKNQVSLTCLVKGFYPSDIAVEWESNGQPENNYKTTPPVLDSDGSFFLYSKLTVDKSRWQQGNVFSCSVMHEALHNHYTQKSLSLSPGK

SEQ ID NO: 21 - protein, 10 aa, synthetic construct
  REGION 1..10: note = Description of Artificial Sequence: Synthetic peptide
GGGGSGGGGS

SEQ ID NO: 22 - protein, 22 aa, unidentified
  REGION 1..22: note = Description of Unknown: Native sequence
MGRGLLRGLWPLHIVLWTRIAS

SEQ ID NO: 23 - protein, 22 aa, unidentified
  REGION 1..22: note = Description of Unknown: Tissue plasminogen activator sequence
MDAMKRGLCCVLLLCGAVFVSP

SEQ ID NO: 24 - protein, 21 aa, Apis sp.
MKFLVNVALVFMVVYISYIYA

SEQ ID NO: 25 - protein, 26 aa, synthetic construct
  REGION 1..26: note = Description of Artificial Sequence: Synthetic peptide
TGGGGSGGGGSGGGGSGGGGSGGGGS

SEQ ID NO: 26 - protein, 31 aa, synthetic construct
  REGION 1..31: note = Description of Artificial Sequence: Synthetic polypeptide
TGGGGSGGGGSGGGGSGGGGSGGGGSGGGGS

SEQ ID NO: 27 - protein, 137 aa, Homo sapiens
TIPPHVQKSVNNDMIVTDNNGAVKFPQLCKFCDVRFSTCDNQKSCMSNCSITSICEKPQEVCVAVWRKNDENITLETVCHDPKLPYHDFILEDAASPKCIMKEKKKPGETFFMCSCSSDECNDNIIFSEEYNTSNPD

SEQ ID NO: 28 - protein, 131 aa, synthetic construct
  REGION 1..131: note = Description of Artificial Sequence: Synthetic polypeptide
QKSVNNDMIVTDNNGAVKFPQLCKFCDVRFSTCDNQKSCMSNCSITSICEKPQEVCVAVWRKNDENITLETVCHDPKLPYHDFILEDAASPKCIMKEKKKPGETFFMCSCSSDECNDNIIFSEEYNTSNPD

SEQ ID NO: 29 - protein, 125 aa, synthetic construct
  REGION 1..125: note = Description of Artificial Sequence: Synthetic polypeptide
DMIVTDNNGAVKFPQLCKFCDVRFSTCDNQKSCMSNCSITSICEKPQEVCVAVWRKNDENITLETVCHDPKLPYHDFILEDAASPKCIMKEKKKPGETFFMCSCSSDECNDNIIFSEEYNTSNPD

SEQ ID NO: 30 - protein, 131 aa, synthetic construct
  REGION 1..131: note = Description of Artificial Sequence: Synthetic polypeptide
TIPPHVQKSVNNDMIVTDNNGAVKFPQLCKFCDVRFSTCDNQKSCMSNCSITSICEKPQEVCVAVWRKNDENITLETVCHDPKLPYHDFILEDAASPKCIMKEKKKPGETFFMCSCSSDECNDNIIFSEEY

SEQ ID NO: 31 - protein, 125 aa, synthetic construct
  REGION 1..125: note = Description of Artificial Sequence: Synthetic polypeptide
QKSVNNDMIVTDNNGAVKFPQLCKFCDVRFSTCDNQKSCMSNCSITSICEKPQEVCVAVWRKNDENITLETVCHDPKLPYHDFILEDAASPKCIMKEKKKPGETFFMCSCSSDECNDNIIFSEEY

SEQ ID NO: 32 - protein, 119 aa, synthetic construct
  REGION 1..119: note = Description of Artificial Sequence: Synthetic polypeptide
DMIVTDNNGAVKFPQLCKFCDVRFSTCDNQKSCMSNCSITSICEKPQEVCVAVWRKNDENITLETVCHDPKLPYHDFILEDAASPKCIMKEKKKPGETFFMCSCSSDECNDNIIFSEEY

SEQ ID NO: 33 - protein, 156 aa, synthetic construct
  REGION 1..156: note = Description of Artificial Sequence: Synthetic polypeptide
QKSDVEMEAQKDEIICPSCNRTAHPLRHINNDMIVTDNNGAVKFPQLCKFCDVRFSTCDNQKSCMSNCSITSICEKPQEVCVAVWRKNDENITLETVCHDPKLPYHDFILEDAASPKCIMKEKKKPGETFFMCSCSSDECNDNIIFSEEYNTSNPD

SEQ ID NO: 34 - protein, 156 aa, synthetic construct
  REGION 1..156: note = Description of Artificial Sequence: Synthetic polypeptide
TIPPHVQKSDVEMEAQKDEIICPSCNRTAHPLRHINNDMIVTDNNGAVKFPQLCKFCDVRFSTCDNQKSCMSNCSITSICEKPQEVCVAVWRKNDENITLETVCHDPKLPYHDFILEDAASPKCIMKEKKKPGETFFMCSCSSDECNDNIIFSEEY

SEQ ID NO: 35 - protein, 150 aa, synthetic construct
  REGION 1..150: note = Description of Artificial Sequence: Synthetic polypeptide
QKSDVEMEAQKDEIICPSCNRTAHPLRHINNDMIVTDNNGAVKFPQLCKFCDVRFSTCDNQKSCMSNCSITSICEKPQEVCVAVWRKNDENITLETVCHDPKLPYHDFILEDAASPKCIMKEKKKPGETFFMCSCSSDECNDNIIFSEEY

SEQ ID NO: 36 - protein, 137 aa, synthetic construct
  REGION 1..137: note = Description of Artificial Sequence: Synthetic polypeptide
TIPPHVQKSVNNDMIVTDNNGAVKFPQLCKFCDVRFSTCDNQKSCMSNCSITSICEKPQEVCVAVWRKNDENITLETVCHDPKLPYHKFILEDAASPKCIMKEKKKPGETFFMCSCSSDECNDNIIFSEEYNTSNPD

SEQ ID NO: 37 - protein, 162 aa, synthetic construct
  REGION 1..162: note = Description of Artificial Sequence: Synthetic polypeptide
TIPPHVQKSDVEMEAQKDEIICPSCNRTAHPLRHINNDMIVTDNNGAVKFPQLCKFCDVRFSTCDNQKSCMSNCSITSICEKPQEVCVAVWRKNDENITLETVCHDPKLPYHKFILEDAASPKCIMKEKKKPGETFFMCSCSSDECNDNIIFSEEYNTSNPD

SEQ ID NO: 38 - protein, 131 aa, synthetic construct
  REGION 1..131: note = Description of Artificial Sequence: Synthetic polypeptide
TIPPHVQKSVNNDMIVTDNNGAVKFPQLCKFCDVRFSTCDNQKSCMSDCSITSICEKPQEVCVAVWRKNDENITLETVCHDPKLPYHDFILEDAASPKCIMKEKKKPGETFFMCSCSSDECNDNIIFSEEY

SEQ ID NO: 39 - protein, 156 aa, synthetic construct
  REGION 1..156: note = Description of Artificial Sequence: Synthetic polypeptide
TIPPHVQKSDVEMEAQKDEIICPSCNRTAHPLRHINNDMIVTDNNGAVKFPQLCKFCDVRFSTCDNQKSCMSDCSITSICEKPQEVCVAVWRKNDENITLETVCHDPKLPYHDFILEDAASPKCIMKEKKKPGETFFMCSCSSDECNDNIIFSEEY

SEQ ID NO: 40 - protein, 36 aa, synthetic construct
  REGION 1..36: note = Description of Artificial Sequence: Synthetic polypeptide
TGGGGSGGGGSGGGGSGGGGSGGGGSGGGGSGGGGS

SEQ ID NO: 41 - protein, 36 aa, Homo sapiens
GRCKIRHIGSNNRLQRSTCQNTGWESAHVMKTPGFR

SEQ ID NO: 42 - protein, 223 aa, Homo sapiens
VECPPCPAPPVAGPSVFLFPPKPKDTLMISRTPEVTCVVVDVSHEDPEVQFNWYVDGVEVHNAKTKPREEQFNSTFRVVSVLTVVHQDWLNGKEYKCKVSNKGLPAPIEKTISKTKGQPREPQVYTLPPSREEMTKNQVSLTCLVKGFYPSDIAVEWESNGQPENNYKTTPPMLDSDGSFFLYSKLTVDKSRWQQGNVFSCSVMHEALHNHYTQKSLSLSPGK

SEQ ID NO: 43 - protein, 233 aa, Homo sapiens
GGPKSCDKTHTCPPCPAPELLGGPSVFLFPPKPKDTLMISRTPEVTCVVVDVSHEDPEVKFNWYVDGVEVHNAKTKPREEQYNSTYRVVSVLTVLHQDWLNGKEYKCKVSNKALPAPIEKTISKAKGQPREPQVYTLPPSREEMTKNQVSLTCLVKGFYPSDIAVEWESNGQPENNYKTTPPVLDSDGSFFLYSKLTVDKSRWQQGNVFSCSVMHEALHNHYTQKSLSLSPGK

SEQ ID NO: 44 - protein, 437 aa, synthetic construct
  REGION 1..437: note = Description of Artificial Sequence: Synthetic polypeptide
MDAMKRGLCCVLLLCGAVFVSPGATIPPHVQKSDVEMEAQKDEIICPSCNRTAHPLRHINNDMIVTDNNGAVKFPQLCKFCDVRFSTCDNQKSCMSNCSITSICEKPQEVCVAVWRKNDENITLETVCHDPKLPYHDFILEDAASPKCIMKEKKKPGETFFMCSCSSDECNDNIIFSEEYNTSNPDTGGGGSGGGGSGGGGSGGGGSGGGGSTHTCPPCPAPELLGGPSVFLFPPKPKDTLMISRTPEVTCVVVDVSHEDPEVKFNWYVDGVEVHNAKTKPREEQYNSTYRVVSVLTVLHQDWLNGKEYKCKVSNKALPAPIEKTISKAKGQPREPQVYTLPPSREEMTKNQVSLTCLVKGFYPSDIAVEWESNGQPENNYKTTPPVLDSDGSFFLYSKLTVDKSRWQQGNVFSCSVMHEALHNHYTQKSLSLSPGK

SEQ ID NO: 45 - protein, 442 aa, synthetic construct
  REGION 1..442: note = Description of Artificial Sequence: Synthetic polypeptide
MDAMKRGLCCVLLLCGAVFVSPGATIPPHVQKSDVEMEAQKDEIICPSCNRTAHPLRHINNDMIVTDNNGAVKFPQLCKFCDVRFSTCDNQKSCMSNCSITSICEKPQEVCVAVWRKNDENITLETVCHDPKLPYHDFILEDAASPKCIMKEKKKPGETFFMCSCSSDECNDNIIFSEEYNTSNPDTGGGGSGGGGSGGGGSGGGGSGGGGSGGGGSTHTCPPCPAPELLGGPSVFLFPPKPKDTLMISRTPEVTCVVVDVSHEDPEVKFNWYVDGVEVHNAKTKPREEQYNSTYRVVSVLTVLHQDWLNGKEYKCKVSNKALPAPIEKTISKAKGQPREPQVYTLPPSREEMTKNQVSLTCLVKGFYPSDIAVEWESNGQPENNYKTTPPVLDSDGSFFLYSKLTVDKSRWQQGNVFSCSVMHEALHNHYTQKSLSLSPGK

SEQ ID NO: 46 - DNA, 1314 bp, synthetic construct
  misc_feature 1..1314: note = Description of Artificial Sequence: Synthetic polynucleotide
  source 1..1314: mol_type = other DNA
atggatgcaatgaagagagggctctgctgtgtgctgctgctgtgtggagcagtcttcgtttcgcccggcgccacgatcccaccgcacgttcagaagtcggatgtggaaatggaggcccagaaagatgaaatcatctgccccagctgtaataggactgcccatccactgagacatattaataacgacatgatagtcactgacaacaacggtgcagtcaagtttccacaactgtgtaaattttgtgatgtgagattttccacctgtgacaaccagaaatcctgcatgagcaactgcagcatcacctccatctgtgagaagccacaggaagtctgtgtggctgtatggagaaagaatgacgagaacataacactagagacagtttgccatgaccccaagctcccctaccatgactttattctggaagatgctgcttctccaaagtgcattatgaaggaaaaaaaaaagcctggtgagactttcttcatgtgttcctgtagctctgatgagtgcaatgacaacatcatcttctcagaagaatataacaccagcaatcctgacaccggtggaggaggttctggtggtggaggttctggaggtggaggaagtggtggaggtggttctggaggtggtggaagtactcacacatgcccaccgtgcccagcacctgaactcctggggggaccgtcagtcttcctcttccccccaaaacccaaggacaccctcatgatctcccggacccctgaggtcacatgcgtggtggtggacgtgagccacgaagaccctgaggtcaagttcaactggtacgtggacggcgtggaggtgcataatgccaagacaaagccgcgggaggagcagtacaacagcacgtaccgtgtggtcagcgtcctcaccgtcctgcaccaggactggctgaatggcaaggagtacaagtgcaaggtctccaacaaagccctcccagcccccatcgagaaaaccatctccaaagccaaagggcagccccgagaaccacaggtgtacaccctgcccccatcccgggaggagatgaccaagaaccaggtcagcctgacctgcctggtcaaaggcttctatcccagcgacatcgccgtggagtgggagagcaatgggcagccggagaacaactacaagaccacgcctcccgtgctggactccgacggctccttcttcctctatagcaagctcaccgtggacaagagcaggtggcagcaggggaacgtcttctcatgctccgtgatgcatgaggctctgcacaaccactacacgcagaagagcctctccctgtctccgggtaaatga

SEQ ID NO: 47 - DNA, 1329 bp, synthetic construct
  misc_feature 1..1329: note = Description of Artificial Sequence: Synthetic polynucleotide
  source 1..1329: mol_type = other DNA
atggatgcaatgaagagagggctctgctgtgtgctgctgctgtgtggagcagtcttcgtttcgcccggcgccacgatcccaccgcacgttcagaagtcggatgtggaaatggaggcccagaaagatgaaatcatctgccccagctgtaataggactgcccatccactgagacatattaataacgacatgatagtcactgacaacaacggtgcagtcaagtttccacaactgtgtaaattttgtgatgtgagattttccacctgtgacaaccagaaatcctgcatgagcaactgcagcatcacctccatctgtgagaagccacaggaagtctgtgtggctgtatggagaaagaatgacgagaacataacactagagacagtttgccatgaccccaagctcccctaccatgactttattctggaagatgctgcttctccaaagtgcattatgaaggaaaaaaaaaagcctggtgagactttcttcatgtgttcctgtagctctgatgagtgcaatgacaacatcatcttctcagaagaatataacaccagcaatcctgacaccggtggaggtggaagtggtggaggaggttctggtggtggaggttctggaggtggaggaagtggtggaggtggttctggaggtggtggaagtactcacacatgcccaccgtgcccagcacctgaactcctggggggaccgtcagtcttcctcttccccccaaaacccaaggacaccctcatgatctcccggacccctgaggtcacatgcgtggtggtggacgtgagccacgaagaccctgaggtcaagttcaactggtacgtggacggcgtggaggtgcataatgccaagacaaagccgcgggaggagcagtacaacagcacgtaccgtgtggtcagcgtcctcaccgtcctgcaccaggactggctgaatggcaaggagtacaagtgcaaggtctccaacaaagccctcccagcccccatcgagaaaaccatctccaaagccaaagggcagccccgagaaccacaggtgtacaccctgcccccatcccgggaggagatgaccaagaaccaggtcagcctgacctgcctggtcaaaggcttctatcccagcgacatcgccgtggagtgggagagcaatgggcagccggagaacaactacaagaccacgcctcccgtgctggactccgacggctccttcttcctctatagcaagctcaccgtggacaagagcaggtggcagcaggggaacgtcttctcatgctccgtgatgcatgaggctctgcacaaccactacacgcagaagagcctctccctgtctccgggtaaatga

SEQ ID NO: 48 - protein, 408 aa, synthetic construct
  REGION 1..408: note = Description of Artificial Sequence: Synthetic polypeptide
TIPPHVQKSDVEMEAQKDEIICPSCNRTAHPLRHINNDMIVTDNNGAVKFPQLCKFCDVRFSTCDNQKSCMSNCSITSICEKPQEVCVAVWRKNDENITLETVCHDPKLPYHDFILEDAASPKCIMKEKKKPGETFFMCSCSSDECNDNIIFSEEYNTSNPDTGGGGSGGGGSGGGGSGGGGSTHTCPPCPAPELLGGPSVFLFPPKPKDTLMISRTPEVTCVVVDVSHEDPEVKFNWYVDGVEVHNAKTKPREEQYNSTYRVVSVLTVLHQDWLNGKEYKCKVSNKALPAPIEKTISKAKGQPREPQVYTLPPSREEMTKNQVSLTCLVKGFYPSDIAVEWESNGQPENNYKTTPPVLDSDGSFFLYSKLTVDKSRWQQGNVFSCSVMHEALHNHYTQKSLSLSPGK

SEQ ID NO: 49 - protein, 162 aa, Homo sapiens; identical to SEQ ID NO: 18

SEQ ID NO: 50 - protein, 410 aa, synthetic construct
  REGION 1..410: note = Description of Artificial Sequence: Synthetic polypeptide
GATIPPHVQKSDVEMEAQKDEIICPSCNRTAHPLRHINNDMIVTDNNGAVKFPQLCKFCDVRFSTCDNQKSCMSNCSITSICEKPQEVCVAVWRKNDENITLETVCHDPKLPYHDFILEDAASPKCIMKEKKKPGETFFMCSCSSDECNDNIIFSEEYNTSNPDTGGGGSGGGGSGGGGSGGGGSTHTCPPCPAPELLGGPSVFLFPPKPKDTLMISRTPEVTCVVVDVSHEDPEVKFNWYVDGVEVHNAKTKPREEQYNSTYRVVSVLTVLHQDWLNGKEYKCKVSNKALPAPIEKTISKAKGQPREPQVYTLPPSREEMTKNQVSLTCLVKGFYPSDIAVEWESNGQPENNYKTTPPVLDSDGSFFLYSKLTVDKSRWQQGNVFSCSVMHEALHNHYTQKSLSLSPGK

SEQ ID NO: 51 - protein, 408 aa, synthetic construct; identical to SEQ ID NO: 48
  REGION 1..408: note = Description of Artificial Sequence: Synthetic polypeptide

SEQ ID NO: 52 - protein, 409 aa, synthetic construct
  REGION 1..409: note = Description of Artificial Sequence: Synthetic polypeptide
ATIPPHVQKSDVEMEAQKDEIICPSCNRTAHPLRHINNDMIVTDNNGAVKFPQLCKFCDVRFSTCDNQKSCMSNCSITSICEKPQEVCVAVWRKNDENITLETVCHDPKLPYHDFILEDAASPKCIMKEKKKPGETFFMCSCSSDECNDNIIFSEEYNTSNPDTGGGGSGGGGSGGGGSGGGGSTHTCPPCPAPELLGGPSVFLFPPKPKDTLMISRTPEVTCVVVDVSHEDPEVKFNWYVDGVEVHNAKTKPREEQYNSTYRVVSVLTVLHQDWLNGKEYKCKVSNKALPAPIEKTISKAKGQPREPQVYTLPPSREEMTKNQVSLTCLVKGFYPSDIAVEWESNGQPENNYKTTPPVLDSDGSFFLYSKLTVDKSRWQQGNVFSCSVMHEALHNHYTQKSLSLSPGK

SEQ ID NO: 53 - protein, 407 aa, synthetic construct
  REGION 1..407: note = Description of Artificial Sequence: Synthetic polypeptide
IPPHVQKSDVEMEAQKDEIICPSCNRTAHPLRHINNDMIVTDNNGAVKFPQLCKFCDVRFSTCDNQKSCMSNCSITSICEKPQEVCVAVWRKNDENITLETVCHDPKLPYHDFILEDAASPKCIMKEKKKPGETFFMCSCSSDECNDNIIFSEEYNTSNPDTGGGGSGGGGSGGGGSGGGGSTHTCPPCPAPELLGGPSVFLFPPKPKDTLMISRTPEVTCVVVDVSHEDPEVKFNWYVDGVEVHNAKTKPREEQYNSTYRVVSVLTVLHQDWLNGKEYKCKVSNKALPAPIEKTISKAKGQPREPQVYTLPPSREEMTKNQVSLTCLVKGFYPSDIAVEWESNGQPENNYKTTPPVLDSDGSFFLYSKLTVDKSRWQQGNVFSCSVMHEALHNHYTQKSLSLSPGK

SEQ ID NO: 54 - protein, 406 aa, synthetic construct
  REGION 1..406: note = Description of Artificial Sequence: Synthetic polypeptide
PPHVQKSDVEMEAQKDEIICPSCNRTAHPLRHINNDMIVTDNNGAVKFPQLCKFCDVRFSTCDNQKSCMSNCSITSICEKPQEVCVAVWRKNDENITLETVCHDPKLPYHDFILEDAASPKCIMKEKKKPGETFFMCSCSSDECNDNIIFSEEYNTSNPDTGGGGSGGGGSGGGGSGGGGSTHTCPPCPAPELLGGPSVFLFPPKPKDTLMISRTPEVTCVVVDVSHEDPEVKFNWYVDGVEVHNAKTKPREEQYNSTYRVVSVLTVLHQDWLNGKEYKCKVSNKALPAPIEKTISKAKGQPREPQVYTLPPSREEMTKNQVSLTCLVKGFYPSDIAVEWESNGQPENNYKTTPPVLDSDGSFFLYSKLTVDKSRWQQGNVFSCSVMHEALHNHYTQKSLSLSPGK

SEQ ID NO: 55 - protein, 405 aa, synthetic construct
  REGION 1..405: note = Description of Artificial Sequence: Synthetic polypeptide
PHVQKSDVEMEAQKDEIICPSCNRTAHPLRHINNDMIVTDNNGAVKFPQLCKFCDVRFSTCDNQKSCMSNCSITSICEKPQEVCVAVWRKNDENITLETVCHDPKLPYHDFILEDAASPKCIMKEKKKPGETFFMCSCSSDECNDNIIFSEEYNTSNPDTGGGGSGGGGSGGGGSGGGGSTHTCPPCPAPELLGGPSVFLFPPKPKDTLMISRTPEVTCVVVDVSHEDPEVKFNWYVDGVEVHNAKTKPREEQYNSTYRVVSVLTVLHQDWLNGKEYKCKVSNKALPAPIEKTISKAKGQPREPQVYTLPPSREEMTKNQVSLTCLVKGFYPSDIAVEWESNGQPENNYKTTPPVLDSDGSFFLYSKLTVDKSRWQQGNVFSCSVMHEALHNHYTQKSLSLSPGK

SEQ ID NO: 56 - protein, 404 aa, synthetic construct
  REGION 1..404: note = Description of Artificial Sequence: Synthetic polypeptide
HVQKSDVEMEAQKDEIICPSCNRTAHPLRHINNDMIVTDNNGAVKFPQLCKFCDVRFSTCDNQKSCMSNCSITSICEKPQEVCVAVWRKNDENITLETVCHDPKLPYHDFILEDAASPKCIMKEKKKPGETFFMCSCSSDECNDNIIFSEEYNTSNPDTGGGGSGGGGSGGGGSGGGGSTHTCPPCPAPELLGGPSVFLFPPKPKDTLMISRTPEVTCVVVDVSHEDPEVKFNWYVDGVEVHNAKTKPREEQYNSTYRVVSVLTVLHQDWLNGKEYKCKVSNKALPAPIEKTISKAKGQPREPQVYTLPPSREEMTKNQVSLTCLVKGFYPSDIAVEWESNGQPENNYKTTPPVLDSDGSFFLYSKLTVDKSRWQQGNVFSCSVMHEALHNHYTQKSLSLSPGK

SEQ ID NO: 57 - protein, 10 aa, synthetic construct
  REGION 1..10: note = Description of Artificial Sequence: Synthetic peptide
  REGION 1..10: note = See specification as filed for detailed description of substitutions and preferred embodiments
GGGGSGGGGS

SEQ ID NO: 58 - protein, 15 aa, synthetic construct
  REGION 1..15: note = Description of Artificial Sequence: Synthetic peptide
  REGION 1..15: note = See specification as filed for detailed description of substitutions and preferred embodiments
GGGGSGGGGSGGGGS

SEQ ID NO: 59 - protein, 20 aa, synthetic construct
  REGION 1..20: note = Description of Artificial Sequence: Synthetic peptide
  REGION 1..20: note = See specification as filed for detailed description of substitutions and preferred embodiments
GGGGSGGGGSGGGGSGGGGS

SEQ ID NO: 60 - protein, 25 aa, synthetic construct
  REGION 1..25: note = Description of Artificial Sequence: Synthetic peptide
  REGION 1..25: note = See specification as filed for detailed description of substitutions and preferred embodiments
GGGGSGGGGSGGGGSGGGGSGGGGS

SEQ ID NO: 61 - protein, 6 aa, synthetic construct
  REGION 1..6: note = Description of Artificial Sequence: Synthetic 6xHis tag
HHHHHH

SEQ ID NO: 62 - protein, 17 aa, synthetic construct
  REGION 1..17: note = Description of Artificial Sequence: Synthetic peptide
NTSNPDTGGGTHTCPPC

SEQ ID NO: 63 - protein, 24 aa, synthetic construct
  REGION 1..24: note = Description of Artificial Sequence: Synthetic peptide
NTSNPDTGGGGSGGGGSTHTCPPC

SEQ ID NO: 64 - protein, 29 aa, synthetic construct
  REGION 1..29: note = Description of Artificial Sequence: Synthetic peptide
NTSNPDTGGGGSGGGGSGGGGSTHTCPPC

SEQ ID NO: 65 - protein, 34 aa, synthetic construct
  REGION 1..34: note = Description of Artificial Sequence: Synthetic polypeptide
NTSNPDTGGGGSGGGGSGGGGSGGGGSTHTCPPC

SEQ ID NO: 66 - protein, 23 aa, synthetic construct
  REGION 1..23: note = Description of Artificial Sequence: Synthetic peptide
NTSNPDTGGGPKSCDKTHTCPPC